European Patent Specification EP 3 863 682 B1, published May 17, 2023. Title: CODON-OPTIMIZED TRANSGENE FOR THE TREATMENT OF PROGRESSIVE FAMILIAR INTRAHEPATIC CHOLESTASIS TYPE 3 (PFIC3). Applicant: VIVET THERAPEUTICS. The sequence listing filed with the application follows.

SEQUENCE LISTING (10 sequences)

SEQ ID NO: 1 - DNA, 3840 bp, artificial sequence
  Codon-optimized sequence encoding MDR3 isoform A
atggatctggaggccgccaagaacggcaccgcctggagacccacaagcgccgagggcgacttcgagctgggcatcagctccaagcagaagagaaagaagaccaagacagtgaagatgatcggcgtgctgacactgttcaggtactccgactggcaggataagctgtttatgtctctgggcaccatcatggcaatcgcccacggcagcggcctgcctctgatgatgatcgtgttcggcgagatgaccgacaagtttgtggatacagccggcaatttctcctttcccgtgaacttctctctgagcctgctgaaccctggcaagatcctggaggaggagatgacaagatatgcctactattactctggcctgggagcaggcgtgctggtggcagcatacatccaggtgagcttctggaccctggcagcaggccggcagatcagaaagatcaggcagaagttctttcacgccatcctgcgccaggagatcggctggtttgacatcaatgataccacagagctgaacacccggctgacagacgacatctctaagatcagcgagggcatcggcgataaagtgggcatgttctttcaggccgtggccacattctttgccggcttcatcgtgggctttatcaggggctggaagctgaccctggtcatcatggccatctctccaatcctgggcctgagcgccgccgtgtgggcaaagatcctgtccgccttctctgacaaggagctggccgcctacgccaaggcaggagcagtggcagaggaggccctgggcgccatccgcaccgtgatcgcctttggcggccagaataaggagctggagcggtatcagaagcacctggagaacgccaaggagatcggcatcaagaaggccatctccgccaatatctctatgggcatcgccttcctgctgatctatgccagctacgccctggccttttggtatggcagcaccctggtcatcagcaaggagtacaccatcggcaatgccatgacagtgttctttagcatcctgatcggagccttctccgtgggacaggcagcaccatgcatcgacgccttcgccaacgccagaggcgcagcctacgtgatctttgacatcatcgataacaatccaaagatcgactccttttctgagcggggccacaagcccgattccatcaagggcaatctggagttcaacgacgtgcactttagctatccctcccgcgccaatgtgaagatcctgaagggcctgaacctgaaggtgcagtccggacagacagtggccctggtgggctctagcggatgcggcaagtctaccacagtgcagctgatccagcggctgtatgacccagatgagggcaccatcaacatcgacggccaggacatccgcaacttcaatgtgaactacctgcgggagatcatcggcgtggtgtctcaggagcccgtgctgtttagcaccacaatcgccgagaatatctgttatggccgcggcaacgtgacaatggatgagatcaagaaggccgtgaaggaggccaatgcctacgagttcatcatgaagctgccccagaagtttgacaccctggtgggagagagaggcgcccagctgagcggaggccagaagcagaggatcgccatcgccagagccctggtgaggaaccctaagatcctgctgctggacgaggccacctccgccctggatacagagtctgaggcagaggtgcaggccgccctggataaggcccgcgagggacggaccacaatcgtgatcgcccacagactgagcacagtgaggaatgccgacgtgatcgccggcttcgaggatggcgtgatcgtggagcagggcagccactccgagctgatgaagaaggagggcgtgtacttcaagctggtgaacatgcagacctctggcagccagatccagtccgaggagtttgagctgaatgacgagaaggcagcaacaaggatggcacctaacggatggaagagcagactgttcaggcactccacccagaagaatctgaagaactctcagatgtgccagaagagcctggacgtggaaaccgatggactggaggcaaatgtgccacccgtgagcttcctgaaggtgctgaagctgaacaagacagagtggccatattttgtggtgggcaccgtgtgcgcaatcgcaaatggcggcctgcagccagccttcagcgtgatcttttccgagatcatcgccatcttcggccctggcgacgatgccgtgaagcagcagaagtgtaacatcttttccctgatcttcctgtttctgggcatcatctctttctttaccttctttctgcagggcttcacatttggcaaggccggcgagatcctgacacggagactgagaagcatggccttcaaggccatgctgaggcaggatatgtcctggtttgacgatcacaagaacagcaccggcgccctgtccaccagactggcaacagacgcagcacaggtgcagggagcaaccggcacaaggctggccctgatcgcccagaatatcgccaacctgggcacaggcatcatcatctctttcatctacggctggcagctgaccctgctgctgctggcagtggtgccaatcatcgccgtgagcggcatcgtggagatgaagctgctggccggcaatgccaagagagacaagaaggagctggaggcagcaggcaagatcgcaaccgaggccatcgagaacatccgcaccgtggtgagcctgacacaggagcggaagttcgagtccatgtatgtggagaagctgtatggcccttaccgcaattccgtgcagaaggcccacatctacggcatcaccttttccatctctcaggctttcatgtatttttcttacgccggctgcttccggtttggcgcctatctgatcgtgaacggccacatgaggttccgcgatgtgatcctggtgttctctgccatcgtgtttggagcagtggccctgggacacgcctcctcttttgcccctgactatgcaaaggcaaagctgtccgccgcacacctgttcatgctgtttgagagacagcctctgatcgatagctactccgaggagggcctgaagccagacaagttcgagggcaatatcacattcaacgaggtggtgtttaattatccaaccagggccaacgtgcccgtgctgcagggcctgagcctggaggtgaagaagggacagacactggccctggtgggcagctccggatgcggcaagtccaccgtggtgcagctgctggagagattctacgaccctctggcaggcaccgtgctgctggatggacaggaggccaagaagctgaatgtgcagtggctgagagcccagctgggcatcgtgtctcaggagccaatcctgttcgattgtagcatcgccgagaatatcgcctacggcgacaactctagggtggtgagccaggatgagatcgtgagcgccgcaaaggcagcaaacatccacccttttatcgagaccctgccacacaagtatgagacacgcgtgggcgacaagggcacccagctgtccggaggacagaagcagaggatcgcaatcgcccgcgccctgatcaggcagccccagatcctgctgctggatgaagccacctccgccctggacacagagtctgagaaggtggtgcaggaggccctggacaaagcccgcgagggacggacatgtattgtcattgctcacagactgagcaccatccagaatgccgacctgatcgtggtgttccagaacggcagggtgaaggagcacggcacacaccagcagctgctggcccagaagggcatctacttttctatggtgagcgtgcaggccggcacccagaacctgtag

SEQ ID NO: 2 - DNA, 3840 bp, artificial sequence
  Codon-optimized sequence encoding MDR3 isoform A #2
atggatctggaagctgccaaaaatggcacagcttggaggcccacctctgctgaaggggattttgagctgggcatcagcagcaagcagaagagaaaaaagaccaagacagtgaagatgattggggtgctgaccctgttcagatactctgactggcaggacaagctgttcatgagcctgggcaccatcatggccattgctcatggttctggcctgcctctgatgatgattgtgtttggggagatgacagacaagtttgtggacacagctggcaacttcagcttccctgtgaacttcagcctgagcctgctgaaccctggcaagatcctggaagaggaaatgaccagatacgcctactactactctggccttggagctggtgtcctggtggctgcctatatccaggtgtccttttggaccctggctgctggcagacagatcagaaagatcaggcagaaattcttccatgccatcctgaggcaagagattggatggtttgacatcaatgacaccacagagctgaacaccaggctgacagatgacatcagcaagatctctgaaggcattggggacaaagtggggatgttcttccaggctgtggccaccttctttgctggcttcattgtgggctttatcagaggctggaaactgaccctggtcatcatggctatcagccccatcctgggactgtctgctgctgtgtgggccaaaatcctgtctgccttctctgacaaagaactggcagcctatgccaaggctggtgctgtggctgaagaagccctgggagccatcagaacagtgattgcctttggagggcagaacaaagagctggaaagataccagaaacacctggaaaatgccaaagagataggcatcaagaaggccatctctgccaacatcagcatgggcattgcctttctgctcatctatgccagctatgccctggccttttggtatggcagcaccctggttatcagcaaagagtacaccattggcaacgccatgacagtgttcttcagcatcctgattggagccttttctgttggccaggctgccccttgcattgatgcctttgctaatgccagaggggctgcttatgtgatctttgacattattgacaacaaccccaagattgacagcttctctgagagaggccacaagcctgacagcatcaagggcaaccttgagttcaatgatgtgcacttcagctaccccagcagggccaatgtgaaaatcctgaagggcctgaacctgaaggtgcagtctggacagacagtggcccttgtgggatcttctggctgtggcaagagcaccacagtgcagctgatccagagactgtatgaccctgatgagggcacaatcaacattgatggccaggacatcagaaacttcaatgtgaactacctgagggaaatcataggggttgtgtcccaagagcctgtgctgttcagcaccaccattgctgagaacatctgctatggcaggggcaatgtcacaatggatgagatcaagaaagctgtgaaagaggccaatgcctatgagttcatcatgaagctgccccagaagtttgacacccttgttggagaaagaggggcccagctgtctggtggccagaagcagagaattgccattgccagggctcttgtcagaaaccctaagatcctgctgctggatgaggccacatctgccctggatacagagtctgaggcagaggtgcaggctgcactggataaggctagagagggaagaacaaccattgtgattgcccacagactgagcacagtcagaaatgcagatgtgattgcaggctttgaggatggggtcatagtggaacagggcagccactctgagctgatgaagaaagaaggggtgtacttcaagctggtcaacatgcagaccagtggcagccagatccagtctgaggaatttgagctgaatgatgagaaggctgccaccagaatggcccctaatggctggaagtctaggctgtttagacacagcacccagaagaacctcaagaacagccagatgtgccagaaaagcctggatgttgagacagatggcctggaagccaatgtgcctcctgtgtccttcctgaaagtgctgaagctgaacaagacagagtggccctactttgttgtgggcacagtgtgtgccattgcaaatggtggcctgcagccagctttctctgtgatcttctctgaaatcattgccatctttggccctggggatgatgctgtgaagcagcagaagtgcaatatcttttccctgatcttcctgttcctggggatcatcagtttcttcacattctttctgcaaggcttcacctttggcaaggctggggagatcctgactagaaggctgagatctatggccttcaaagccatgctgagacaggacatgtcttggtttgatgaccacaagaactccacaggggccctgagcacaagactggctacagatgctgctcaggtgcagggtgctacaggcactagactggccctgattgcacagaacattgccaaccttggcacaggcatcatcattagcttcatctatggctggcagctgacactgctcctgctggctgttgtgcccatcattgcagtgtctggcattgtggaaatgaagttgctggctggcaatgccaagagggacaagaaagagcttgaggcagcaggcaagattgccacagaggccattgagaatatcaggacagtggtgtctctgacccaagaaagaaagtttgagtctatgtatgtggaaaagctgtatgggccctataggaactctgtgcaaaaggcccacatctatgggatcaccttctccatcagccaggctttcatgtactttagctatgctggctgcttcagatttggggcctacctgattgtgaatggccacatgagattcagggatgtgatcctggtgttttctgccattgtctttggagctgtggctctgggccatgcctctagctttgcccctgactatgccaaagccaaactgtctgcagcccacctgttcatgctgtttgagagacagcccctgattgactcctactctgaggaaggactgaagcctgataagtttgagggcaacatcaccttcaatgaggtggtgttcaactaccctaccagagctaatgtgccagtgctgcagggactctccctggaagtgaagaaagggcagactctggctcttgtgggcagctcaggatgtggcaagtctacagtggtgcagctgctggaaaggttctatgatcccctggcaggcacagtgctgttggatggccaagaggctaaaaagctgaatgtgcagtggctgagagcacagctgggaattgtgtctcaagaacccatcctgtttgactgcagcatagcagagaacatagcctatggggacaactccagagtggtttctcaggatgagattgtctctgctgccaaggcagccaacattcaccccttcattgagacactgccccacaaatatgagacaagagtgggagacaagggaacccagctcagtggtggacagaaacaaaggattgctatagctagggccctgatcagacagcctcagattctgctccttgatgaagcaacctctgctctggacactgaatctgagaaggtggtgcaagaggccctggacaaagccagagagggtagaacctgcattgtcattgctcacaggctgtctaccatccagaatgctgatctgattgtggtgttccagaatgggagagtgaaagagcatggcacccaccagcaactgctggcccagaagggcatctacttcagcatggtgtctgtgcaggcagggacccagaacctgtaa

SEQ ID NO: 3 - DNA, 56 bp, artificial sequence
  Synthetic poly A sequence
aataaagacctcttattttcattcatcaggtgtggttggtttttttgtgtgggggc

SEQ ID NO: 4 - DNA, 4598 bp, artificial sequence
  recombinant AAV vector comprising codon-optimized sequence encoding MDR3 isoform A
cctgcaggcagctgcgcgctcgctcgctcactgaggccgcccgggcaaagcccgggcgtcgggcgacctttggtcgcccggcctcagtgagcgagcgagcgcgcagagagggagtggccaactccatcactaggggttcctgcggccgcgaattccatggtaccaggcatcaagacacgtgcgccaccccctccaccttggacacaggacgctgtggtttctgagccaggtacaatgactcctttcggtaagtgcagtggaagctgtacactgcccaggcaaagcgtccgggcagcgtaggcgggcgactcagatcccagccagtggacttagcccctgtttgctcctccgataactggggtgaccttggttaatattcaccagcagcctcccccgttgcccctctggatccactgcttaaatacggacgaggacagggccctgtctcctcagcttcaggcaccaccactgacctgggacagtgaaggcctgtcgacggatccgccgccaccatggatctggaggccgccaagaacggcaccgcctggagacccacaagcgccgagggcgacttcgagctgggcatcagctccaagcagaagagaaagaagaccaagacagtgaagatgatcggcgtgctgacactgttcaggtactccgactggcaggataagctgtttatgtctctgggcaccatcatggcaatcgcccacggcagcggcctgcctctgatgatgatcgtgttcggcgagatgaccgacaagtttgtggatacagccggcaatttctcctttcccgtgaacttctctctgagcctgctgaaccctggcaagatcctggaggaggagatgacaagatatgcctactattactctggcctgggagcaggcgtgctggtggcagcatacatccaggtgagcttctggaccctggcagcaggccggcagatcagaaagatcaggcagaagttctttcacgccatcctgcgccaggagatcggctggtttgacatcaatgataccacagagctgaacacccggctgacagacgacatctctaagatcagcgagggcatcggcgataaagtgggcatgttctttcaggccgtggccacattctttgccggcttcatcgtgggctttatcaggggctggaagctgaccctggtcatcatggccatctctccaatcctgggcctgagcgccgccgtgtgggcaaagatcctgtccgccttctctgacaaggagctggccgcctacgccaaggcaggagcagtggcagaggaggccctgggcgccatccgcaccgtgatcgcctttggcggccagaataaggagctggagcggtatcagaagcacctggagaacgccaaggagatcggcatcaagaaggccatctccgccaatatctctatgggcatcgccttcctgctgatctatgccagctacgccctggccttttggtatggcagcaccctggtcatcagcaaggagtacaccatcggcaatgccatgacagtgttctttagcatcctgatcggagccttctccgtgggacaggcagcaccatgcatcgacgccttcgccaacgccagaggcgcagcctacgtgatctttgacatcatcgataacaatccaaagatcgactccttttctgagcggggccacaagcccgattccatcaagggcaatctggagttcaacgacgtgcactttagctatccctcccgcgccaatgtgaagatcctgaagggcctgaacctgaaggtgcagtccggacagacagtggccctggtgggctctagcggatgcggcaagtctaccacagtgcagctgatccagcggctgtatgacccagatgagggcaccatcaacatcgacggccaggacatccgcaacttcaatgtgaactacctgcgggagatcatcggcgtggtgtctcaggagcccgtgctgtttagcaccacaatcgccgagaatatctgttatggccgcggcaacgtgacaatggatgagatcaagaaggccgtgaaggaggccaatgcctacgagttcatcatgaagctgccccagaagtttgacaccctggtgggagagagaggcgcccagctgagcggaggccagaagcagaggatcgccatcgccagagccctggtgaggaaccctaagatcctgctgctggacgaggccacctccgccctggatacagagtctgaggcagaggtgcaggccgccctggataaggcccgcgagggacggaccacaatcgtgatcgcccacagactgagcacagtgaggaatgccgacgtgatcgccggcttcgaggatggcgtgatcgtggagcagggcagccactccgagctgatgaagaaggagggcgtgtacttcaagctggtgaacatgcagacctctggcagccagatccagtccgaggagtttgagctgaatgacgagaaggcagcaacaaggatggcacctaacggatggaagagcagactgttcaggcactccacccagaagaatctgaagaactctcagatgtgccagaagagcctggacgtggaaaccgatggactggaggcaaatgtgccacccgtgagcttcctgaaggtgctgaagctgaacaagacagagtggccatattttgtggtgggcaccgtgtgcgcaatcgcaaatggcggcctgcagccagccttcagcgtgatcttttccgagatcatcgccatcttcggccctggcgacgatgccgtgaagcagcagaagtgtaacatcttttccctgatcttcctgtttctgggcatcatctctttctttaccttctttctgcagggcttcacatttggcaaggccggcgagatcctgacacggagactgagaagcatggccttcaaggccatgctgaggcaggatatgtcctggtttgacgatcacaagaacagcaccggcgccctgtccaccagactggcaacagacgcagcacaggtgcagggagcaaccggcacaaggctggccctgatcgcccagaatatcgccaacctgggcacaggcatcatcatctctttcatctacggctggcagctgaccctgctgctgctggcagtggtgccaatcatcgccgtgagcggcatcgtggagatgaagctgctggccggcaatgccaagagagacaagaaggagctggaggcagcaggcaagatcgcaaccgaggccatcgagaacatccgcaccgtggtgagcctgacacaggagcggaagttcgagtccatgtatgtggagaagctgtatggcccttaccgcaattccgtgcagaaggcccacatctacggcatcaccttttccatctctcaggctttcatgtatttttcttacgccggctgcttccggtttggcgcctatctgatcgtgaacggccacatgaggttccgcgatgtgatcctggtgttctctgccatcgtgtttggagcagtggccctgggacacgcctcctcttttgcccctgactatgcaaaggcaaagctgtccgccgcacacctgttcatgctgtttgagagacagcctctgatcgatagctactccgaggagggcctgaagccagacaagttcgagggcaatatcacattcaacgaggtggtgtttaattatccaaccagggccaacgtgcccgtgctgcagggcctgagcctggaggtgaagaagggacagacactggccctggtgggcagctccggatgcggcaagtccaccgtggtgcagctgctggagagattctacgaccctctggcaggcaccgtgctgctggatggacaggaggccaagaagctgaatgtgcagtggctgagagcccagctgggcatcgtgtctcaggagccaatcctgttcgattgtagcatcgccgagaatatcgcctacggcgacaactctagggtggtgagccaggatgagatcgtgagcgccgcaaaggcagcaaacatccacccttttatcgagaccctgccacacaagtatgagacacgcgtgggcgacaagggcacccagctgtccggaggacagaagcagaggatcgcaatcgcccgcgccctgatcaggcagccccagatcctgctgctggatgaagccacctccgccctggacacagagtctgagaaggtggtgcaggaggccctggacaaagcccgcgagggacggacatgtattgtcattgctcacagactgagcaccatccagaatgccgacctgatcgtggtgttccagaacggcagggtgaaggagcacggcacacaccagcagctgctggcccagaagggcatctacttttctatggtgagcgtgcaggccggcacccagaacctgtagcatatgatatcaataaagacctcttattttcattcatcaggtgtggttggtttttttgtgtgggggctcgagatctgaggaacccctagtgatggaggcggccgcaggaacccctagtgatggagttggccactccctctctgcgcgctcgctcgctcactgaggccgggcgaccaaaggtcgcccgacgcccgggctttgcccgggcggcctcagtgagcgagcgagcgcgcagctgcctgcagg

SEQ ID NO: 5 - DNA, 4598 bp, artificial sequence
  recombinant AAv vector comprising codon-optimized sequence encoding MDR3 isoform A #2
cctgcaggcagctgcgcgctcgctcgctcactgaggccgcccgggcaaagcccgggcgtcgggcgacctttggtcgcccggcctcagtgagcgagcgagcgcgcagagagggagtggccaactccatcactaggggttcctgcggccgcgaattccatggtaccaggcatcaagacacgtgcgccaccccctccaccttggacacaggacgctgtggtttctgagccaggtacaatgactcctttcggtaagtgcagtggaagctgtacactgcccaggcaaagcgtccgggcagcgtaggcgggcgactcagatcccagccagtggacttagcccctgtttgctcctccgataactggggtgaccttggttaatattcaccagcagcctcccccgttgcccctctggatccactgcttaaatacggacgaggacagggccctgtctcctcagcttcaggcaccaccactgacctgggacagtgaaggcctgtcgacggatccgccgccaccatggatctggaagctgccaaaaatggcacagcttggaggcccacctctgctgaaggggattttgagctgggcatcagcagcaagcagaagagaaaaaagaccaagacagtgaagatgattggggtgctgaccctgttcagatactctgactggcaggacaagctgttcatgagcctgggcaccatcatggccattgctcatggttctggcctgcctctgatgatgattgtgtttggggagatgacagacaagtttgtggacacagctggcaacttcagcttccctgtgaacttcagcctgagcctgctgaaccctggcaagatcctggaagaggaaatgaccagatacgcctactactactctggccttggagctggtgtcctggtggctgcctatatccaggtgtccttttggaccctggctgctggcagacagatcagaaagatcaggcagaaattcttccatgccatcctgaggcaagagattggatggtttgacatcaatgacaccacagagctgaacaccaggctgacagatgacatcagcaagatctctgaaggcattggggacaaagtggggatgttcttccaggctgtggccaccttctttgctggcttcattgtgggctttatcagaggctggaaactgaccctggtcatcatggctatcagccccatcctgggactgtctgctgctgtgtgggccaaaatcctgtctgccttctctgacaaagaactggcagcctatgccaaggctggtgctgtggctgaagaagccctgggagccatcagaacagtgattgcctttggagggcagaacaaagagctggaaagataccagaaacacctggaaaatgccaaagagataggcatcaagaaggccatctctgccaacatcagcatgggcattgcctttctgctcatctatgccagctatgccctggccttttggtatggcagcaccctggttatcagcaaagagtacaccattggcaacgccatgacagtgttcttcagcatcctgattggagccttttctgttggccaggctgccccttgcattgatgcctttgctaatgccagaggggctgcttatgtgatctttgacattattgacaacaaccccaagattgacagcttctctgagagaggccacaagcctgacagcatcaagggcaaccttgagttcaatgatgtgcacttcagctaccccagcagggccaatgtgaaaatcctgaagggcctgaacctgaaggtgcagtctggacagacagtggcccttgtgggatcttctggctgtggcaagagcaccacagtgcagctgatccagagactgtatgaccctgatgagggcacaatcaacattgatggccaggacatcagaaacttcaatgtgaactacctgagggaaatcataggggttgtgtcccaagagcctgtgctgttcagcaccaccattgctgagaacatctgctatggcaggggcaatgtcacaatggatgagatcaagaaagctgtgaaagaggccaatgcctatgagttcatcatgaagctgccccagaagtttgacacccttgttggagaaagaggggcccagctgtctggtggccagaagcagagaattgccattgccagggctcttgtcagaaaccctaagatcctgctgctggatgaggccacatctgccctggatacagagtctgaggcagaggtgcaggctgcactggataaggctagagagggaagaacaaccattgtgattgcccacagactgagcacagtcagaaatgcagatgtgattgcaggctttgaggatggggtcatagtggaacagggcagccactctgagctgatgaagaaagaaggggtgtacttcaagctggtcaacatgcagaccagtggcagccagatccagtctgaggaatttgagctgaatgatgagaaggctgccaccagaatggcccctaatggctggaagtctaggctgtttagacacagcacccagaagaacctcaagaacagccagatgtgccagaaaagcctggatgttgagacagatggcctggaagccaatgtgcctcctgtgtccttcctgaaagtgctgaagctgaacaagacagagtggccctactttgttgtgggcacagtgtgtgccattgcaaatggtggcctgcagccagctttctctgtgatcttctctgaaatcattgccatctttggccctggggatgatgctgtgaagcagcagaagtgcaatatcttttccctgatcttcctgttcctggggatcatcagtttcttcacattctttctgcaaggcttcacctttggcaaggctggggagatcctgactagaaggctgagatctatggccttcaaagccatgctgagacaggacatgtcttggtttgatgaccacaagaactccacaggggccctgagcacaagactggctacagatgctgctcaggtgcagggtgctacaggcactagactggccctgattgcacagaacattgccaaccttggcacaggcatcatcattagcttcatctatggctggcagctgacactgctcctgctggctgttgtgcccatcattgcagtgtctggcattgtggaaatgaagttgctggctggcaatgccaagagggacaagaaagagcttgaggcagcaggcaagattgccacagaggccattgagaatatcaggacagtggtgtctctgacccaagaaagaaagtttgagtctatgtatgtggaaaagctgtatgggccctataggaactctgtgcaaaaggcccacatctatgggatcaccttctccatcagccaggctttcatgtactttagctatgctggctgcttcagatttggggcctacctgattgtgaatggccacatgagattcagggatgtgatcctggtgttttctgccattgtctttggagctgtggctctgggccatgcctctagctttgcccctgactatgccaaagccaaactgtctgcagcccacctgttcatgctgtttgagagacagcccctgattgactcctactctgaggaaggactgaagcctgataagtttgagggcaacatcaccttcaatgaggtggtgttcaactaccctaccagagctaatgtgccagtgctgcagggactctccctggaagtgaagaaagggcagactctggctcttgtgggcagctcaggatgtggcaagtctacagtggtgcagctgctggaaaggttctatgatcccctggcaggcacagtgctgttggatggccaagaggctaaaaagctgaatgtgcagtggctgagagcacagctgggaattgtgtctcaagaacccatcctgtttgactgcagcatagcagagaacatagcctatggggacaactccagagtggtttctcaggatgagattgtctctgctgccaaggcagccaacattcaccccttcattgagacactgccccacaaatatgagacaagagtgggagacaagggaacccagctcagtggtggacagaaacaaaggattgctatagctagggccctgatcagacagcctcagattctgctccttgatgaagcaacctctgctctggacactgaatctgagaaggtggtgcaagaggccctggacaaagccagagagggtagaacctgcattgtcattgctcacaggctgtctaccatccagaatgctgatctgattgtggtgttccagaatgggagagtgaaagagcatggcacccaccagcaactgctggcccagaagggcatctacttcagcatggtgtctgtgcaggcagggacccagaacctgtaacatatgatatcaataaagacctcttattttcattcatcaggtgtggttggtttttttgtgtgggggctcgagatctgaggaacccctagtgatggaggcggccgcaggaacccctagtgatggagttggccactccctctctgcgcgctcgctcgctcactgaggccgggcgaccaaaggtcgcccgacgcccgggctttgcccgggcggcctcagtgagcgagcgagcgcgcagctgcctgcagg

SEQ ID NO: 6 - DNA, 255 bp, artificial sequence
  Alpha 1 antitrypsin promoter
cgccaccccctccaccttggacacaggacgctgtggtttctgagccaggtacaatgactcctttcggtaagtgcagtggaagctgtacactgcccaggcaaagcgtccgggcagcgtaggcgggcgactcagatcccagccagtggacttagcccctgtttgctcctccgataactggggtgaccttggttaatattcaccagcagcctcccccgttgcccctctggatccactgcttaaatacggacgaggaca

SEQ ID NO: 7 - DNA, 145 bp, artificial sequence
  Human minimal bile salt export pump (ABCB11) gene promoter
ttcccaagcacactctgtgtttggggttattgctctgagtatgtttctcgtatgtcactgaactgtgcttgggctgcccttagggacattgatccttaggcaaatagataatgttcttgaaaaagtttgaattctgttcagtgct

SEQ ID NO: 8 - DNA, 145 bp, artificial sequence
  Mouse minimal Bile Salt export pump (ABCB11) gene promoter
ggttcctgctttgagtatgttcgacctttcctctcatgtcactgaactgtgctagatctggactttaggccattgacctataagcaaatagatagtgttcttaaaaaagcctgatttctgttcaatgctttattaccatgaaaac

SEQ ID NO: 9 - DNA, 20 bp, artificial sequence
  Forward alpha-1-anti-trypsin promoter primer
ttgctcctccgataactggg

SEQ ID NO: 10 - DNA, 20 bp, artificial sequence
  Reverse alpha-1-anti-trypsin promoter primer
ccctgtcctcgtccgtattt